European Patent Application EP 4 360 656 A2, published May 1, 2024. Title: Polyphosphate-functionalized inorganic nanoparticles as hemostatic compositions and methods of use. Applicant: The Regents of the University of California. Application EP 23218706.2, filed March 7, 2014. The sequence listing filed with the application follows.

SEQUENCE LISTING (9 sequences)

SEQ ID NO: 1 - protein, 4 aa, synthetic construct
  REGION 1..4: note = synthetic amino acid sequence
IEGR

SEQ ID NO: 2 - protein, 5 aa, synthetic construct
  REGION 1..5: note = synthetic amino acid sequence
CREKA

SEQ ID NO: 3 - protein, 7 aa, synthetic construct
  REGION 1..7: note = synthetic amino acid sequence
KLWVLPK

SEQ ID NO: 4 - protein, 12 aa, synthetic construct
  REGION 1..12: note = synthetic amino acid sequence
  MOD_RES 12: note = AMIDATION
NQEQVSPLTGLK

SEQ ID NO: 5 - protein, 14 aa, synthetic construct
  REGION 1..14: note = synthetic amino acid sequence
  MOD_RES 1: note = ACETYLATION
  MOD_RES 14: note = AMIDATION
CGGIEGRGGSGGKG

SEQ ID NO: 6 - protein, 14 aa, synthetic construct
  REGION 1..14: note = synthetic amino acid sequence
  MOD_RES 1: note = ACETYLATION
  MOD_RES 14: note = AMIDATION
CGGIEGRGGKGGKG

SEQ ID NO: 7 - protein, 14 aa, synthetic construct
  REGION 1..14: note = synthetic amino acid sequence
  MOD_RES 14: note = AMIDATION
CGGIEGRGGSGGKG

SEQ ID NO: 8 - protein, 14 aa, synthetic construct
  REGION 1..14: note = synthetic amino acid sequence
  MOD_RES 14: note = AMIDATION
CGGERGIGGSGGKG

SEQ ID NO: 9 - protein, 18 aa, synthetic construct
  REGION 1..18: note = synthetic amino acid sequence
CDGSRPARSGRSAGGKDA